European Patent Application EP 4 445 910 A1, published October 16, 2024. Title: A vaccine composition for inducing an anti-IL-23 antibody. Applicant: 国立大学法人大阪大学. The sequence listing filed with the application follows.

SEQUENCE LISTING (43 sequences)

SEQ ID NO: 1 - protein, 8 aa, Mus musculus
LSSSQQWQ

SEQ ID NO: 2 - protein, 8 aa, Mus musculus
SSSQQWQR

SEQ ID NO: 3 - protein, 8 aa, Mus musculus
SSQQWQRP

SEQ ID NO: 4 - protein, 8 aa, Mus musculus
SQQWQRPL

SEQ ID NO: 5 - protein, 8 aa, Mus musculus
QWQRPLLR

SEQ ID NO: 6 - protein, 8 aa, Homo sapiens
SPSQPWQR

SEQ ID NO: 7 - protein, 8 aa, synthetic construct
  REGION 1..8: note = modified sequence of hIL-23 151-158
APSQPWQR

SEQ ID NO: 8 - protein, 8 aa, synthetic construct
  REGION 1..8: note = modified sequence of hIL-23 151-158
SASQPWQR

SEQ ID NO: 9 - protein, 8 aa, synthetic construct
  REGION 1..8: note = modified sequence of hIL-23 151-158
SPAQPWQR

SEQ ID NO: 10 - protein, 8 aa, synthetic construct
  REGION 1..8: note = modified sequence of hIL-23 151-158
SPSAPWQR

SEQ ID NO: 11 - protein, 8 aa, synthetic construct
  REGION 1..8: note = modified sequence of hIL-23 151-158
SPSQAWQR

SEQ ID NO: 12 - protein, 8 aa, synthetic construct
  REGION 1..8: note = modified sequence of hIL-23 151-158
SPSQPAQR

SEQ ID NO: 13 - protein, 8 aa, synthetic construct
  REGION 1..8: note = modified sequence of hIL-23 151-158
SPSQPWAR

SEQ ID NO: 14 - protein, 8 aa, synthetic construct
  REGION 1..8: note = modified sequence of hIL-23 151-158
SPSQPWQA

SEQ ID NO: 15 - protein, 8 aa, synthetic construct
  REGION 1..8: note = modified sequence of hIL-23 151-158
PWQRPWQR

SEQ ID NO: 16 - protein, 8 aa, synthetic construct
  REGION 1..8: note = modified sequence of hIL-23 151-158
QWQRPWQR

SEQ ID NO: 17 - protein, 8 aa, synthetic construct
  REGION 1..8: note = modified sequence of hIL-23 151-158
SSSQPWQR

SEQ ID NO: 18 - protein, 8 aa, synthetic construct
  REGION 1..8: note = modified sequence of hIL-23 151-158
STSQPWQR

SEQ ID NO: 19 - protein, 8 aa, synthetic construct
  REGION 1..8: note = modified sequence of hIL-23 151-158
SPSQSWQR

SEQ ID NO: 20 - protein, 8 aa, synthetic construct
  REGION 1..8: note = modified sequence of hIL-23 151-158
SPSQTWQR

SEQ ID NO: 21 - protein, 8 aa, synthetic construct
  REGION 1..8: note = modified sequence of hIL-23 151-158
SSSQSWQR

SEQ ID NO: 22 - protein, 8 aa, synthetic construct
  REGION 1..8: note = modified sequence of hIL-23 151-158
SSSQTWQR

SEQ ID NO: 23 - protein, 8 aa, synthetic construct
  REGION 1..8: note = modified sequence of hIL-23 151-158
STSQSWQR

SEQ ID NO: 24 - protein, 8 aa, synthetic construct
  REGION 1..8: note = modified sequence of hIL-23 151-158
STSQTWQR

SEQ ID NO: 25 - protein, 8 aa, synthetic construct
  REGION 1..8: note = modified sequence of hIL-23 151-158
SPSQQWQR

SEQ ID NO: 26 - protein, 8 aa, synthetic construct
  REGION 1..8: note = modified sequence of hIL-23 151-158
STSQQWQR

SEQ ID NO: 27 - protein, 8 aa, synthetic construct
  REGION 1..8: note = modified sequence of hIL-23 151-158
KPSQPWQR

SEQ ID NO: 28 - protein, 8 aa, synthetic construct
  REGION 1..8: note = modified sequence of hIL-23 151-158
SKSQPWQR

SEQ ID NO: 29 - protein, 8 aa, synthetic construct
  REGION 1..8: note = modified sequence of hIL-23 151-158
SPKQPWQR

SEQ ID NO: 30 - protein, 8 aa, synthetic construct
  REGION 1..8: note = modified sequence of hIL-23 151-158
KKSQPWQR

SEQ ID NO: 31 - protein, 7 aa, Homo sapiens
PSQPWQR

SEQ ID NO: 32 - protein, 6 aa, Homo sapiens
SQPWQR

SEQ ID NO: 33 - protein, 5 aa, Homo sapiens
QPWQR

SEQ ID NO: 34 - protein, 8 aa, Homo sapiens
PSQPWQRK

SEQ ID NO: 35 - protein, 7 aa, Homo sapiens
SQPWQRK

SEQ ID NO: 36 - protein, 11 aa, synthetic construct
  REGION 1..11: note = QPWQR-S-QPWQR
QPWQRSQPWQR

SEQ ID NO: 37 - protein, 15 aa, synthetic construct
  REGION 1..15: note = QPWQR-GGGGS-QPWQR
QPWQRGGGGSQPWQR

SEQ ID NO: 38 - protein, 20 aa, synthetic construct
  REGION 1..20: note = AJP001
ELKLIFLHRLKRLRKRLKRK

SEQ ID NO: 39 - protein, 19 aa, synthetic construct
  REGION 1..19: note = UBITh1
ISITEIKGVIVHRIETILF

SEQ ID NO: 40 - protein, 18 aa, synthetic construct
  REGION 1..18: note = UBITh2
KKKIITITRIITIITTID

SEQ ID NO: 41 - protein, 19 aa, synthetic construct
  REGION 1..19: note = UBITh3
ISISEIKGVIVHKIETILF

SEQ ID NO: 42 - protein, 19 aa, synthetic construct
  REGION 1..19: note = UBITh4
ISITEIRTVIVTRIETILF

SEQ ID NO: 43 - protein, 14 aa, Clostridium tetani
QYIKANSKFIGITE